European Patent Application EP 4 248 985 A1, published September 27, 2023. Title: PEPTIDES FOR THE TREATMENT OF RETINITIS PIGMENTOSA. Applicant: CONSEJO SUPERIOR DE INVESTIGACIONES CIENTÍFICAS (CSIC). The sequence listing filed with the application follows.

SEQUENCE LISTING (2 sequences)

SEQ ID NO: 1 - protein, 20 aa, Homo sapiens
  PEPTIDE (1)..(2): Can be any amino acid residue
  PEPTIDE (7)..(20): Can be any amino acid residue
XXRIKPXXXXXXXXXXXXXX

SEQ ID NO: 2 - protein, 15 aa, Homo sapiens
  PEPTIDE (1)..(15): synthetic peptide analog of the Pre Implantation Factor peptide
MVRIKPGSANKPSDD